European Patent Specification EP 4 015 003 B1, published May 10, 2023. Title: IMPROVED ANTIBODY-OLIGONUCLEOTIDE CONJUGATE. Applicant: Sapreme Technologies B.V. Charité - UNIVERSITÄTSMEDIZIN BERLIN. The sequence listing filed with the application follows.

SEQUENCE LISTING (12 sequences)

SEQ ID NO: 1 - DNA, 16 bp, Antisense BNA (HSP27) oligo nucleic acid sequence
ggcacagccagtggcg

SEQ ID NO: 2 - DNA, 18 bp, UBC primer forward sequence
cagccgggatttgggtcg

SEQ ID NO: 3 - DNA, 23 bp, UBC primer reverse sequence
cacgaagatctgcattgtcaagt

SEQ ID NO: 4 - DNA, 20 bp, GUSB primer forward sequence
tgcgtagggacaagaaccac

SEQ ID NO: 5 - DNA, 20 bp, GUSB primer reverse sequence
gggaggggtccaaggatttg

SEQ ID NO: 6 - DNA, 20 bp, IMMT primer forward sequence
aacccacacctgcactttca

SEQ ID NO: 7 - DNA, 20 bp, IMMT primer reverse sequence
ttttcctgttgtgcaaggcg

SEQ ID NO: 8 - DNA, 20 bp, EIF2S2 primer forward sequence
ccacaagtcgtccgagtagg

SEQ ID NO: 9 - DNA, 20 bp, EIF2S2 primer reverse sequence
ggagatgtttgggctgacga

SEQ ID NO: 10 - DNA, 20 bp, HSP27 primer forward sequence
gcagtccaacgagatcacca

SEQ ID NO: 11 - DNA, 20 bp, HSP27 primer reverse sequence
taaggctttacttggcggca

SEQ ID NO: 12 - protein, 18 aa, Customized peptide
SESDDAMFCDAMDESDSK